European Patent Specification EP 4 006 165 B1, published April 29, 2026. Title: MULTIPLEX LIGATION-DEPENDENT PROBE MICROARRAY DETECTION. Applicant: FLASHDX SHENZHEN INC. The sequence listing filed with the application follows.

SEQUENCE LISTING (14 sequences)

SEQ ID NO: 1 - DNA, 24 bp, artificial sequence
  primer
gtcgtgactgggaaaaccctggcg

SEQ ID NO: 2 - DNA, 23 bp, artificial sequence
  primer
agcggataacaatttcacacagg

SEQ ID NO: 3 - DNA, 23 bp, artificial sequence
  the reverse complement
gacaggctgtacctacggtttaa

SEQ ID NO: 4 - DNA, 21 bp, artificial sequence
  the reverse complement
ttgaaacaagccgacgcaacg

SEQ ID NO: 5 - DNA, 25 bp, artificial sequence
  Barcode Index 1
gtaactctacagacggacgtagtca

SEQ ID NO: 6 - DNA, 45 bp, artificial sequence
  The first probe
gtcgtgactgggaaaaccctggcgttgaaacaagccgacgcaacg

SEQ ID NO: 7 - DNA, 71 bp, artificial sequence
  The second probe
gacaggctgtacctacggtttaagtaactctacagacggacgtagtcacctgtgtgaaattgttatccgct

SEQ ID NO: 8 - DNA, 25 bp, artificial sequence
  The surface probe
gtaactctacagacggacgtagtca

SEQ ID NO: 9 - DNA, 22 bp, artificial sequence
  T1'
agatagtcctgagccagcctgt

SEQ ID NO: 10 - DNA, 23 bp, artificial sequence
  T2'
gtggtatctgtaggacgcactgc

SEQ ID NO: 11 - DNA, 25 bp, artificial sequence
  Barcode Index 2
ccctcaacggtatcgcgtcggttgc

SEQ ID NO: 12 - DNA, 47 bp, artificial sequence
  The first probe
gtcgtgactgggaaaaccctggcggtggtatctgtaggacgcactgc

SEQ ID NO: 13 - DNA, 70 bp, artificial sequence
  The second probe
agatagtcctgagccagcctgtccctcaacggtatcgcgtcggttgccctgtgtgaaattgttatccgct

SEQ ID NO: 14 - DNA, 25 bp, artificial sequence
  The surface probe
ccctcaacggtatcgcgtcggttgc